European Patent Specification EP 4 225 805 B1, published June 18, 2025. Title: GROWTH HORMONE FUSION PROTEIN AND PREPARATION METHOD AND USE THEREOF. Applicant: JHM BIOPHARMACEUTICAL (HANGZHOU) Co. , Ltd. The sequence listing filed with the application follows.

SEQUENCE LISTING (6 sequences)

SEQ ID NO: 1 - protein, 192 aa, Artificial Sequence
  Amino acid sequence of growth hormone
  MISC_FEATURE (1)..(1): Xaa represents G, A or S
  MISC_FEATURE (183)..(183): Xaa represents G, A, S, C or deletion
  MISC_FEATURE (190)..(190): Xaa represents G, A, S, C or deletion
XFPTIPLSRLFDNAMLRAHRLHQLAFDTYQEFEEAYIPKEQKYSFLQNPQTSLCFSESIPTPSNREETQQKSNLELLRISLLLIQSWLEPVQFLRSVFANSLVYGASDSNVYDLLKDLEEGIQTLMGRLEDGSPRTGQIFKQTYSKFDTNSHNDDALLKNYGLLYCFRKDMDKVETFLRIVQXRSVEGSXGF

SEQ ID NO: 2 - protein, 228 aa, Artificial Sequence
  Amino acid sequence of first constant region FC segment or second constant region FC segment
  MISC_FEATURE (7)..(7): Xaa represents R, K, D, E or C
  MISC_FEATURE (10)..(10): Xaa represents R, K, D, E or C
  MISC_FEATURE (14)..(14): Xaa represents R, K, D, E or deletion
  MISC_FEATURE (16)..(16): Xaa represents A, R, K, D, E or deletion
  misc_feature (78)..(78): Xaa represents D, E, G, Q or N
  MISC_FEATURE (96)..(96): Xaa represents D, E, G, Q or N
  MISC_FEATURE (147)..(147): Xaa represents G, S or W
  MISC_FEATURE (149)..(149): Xaa represents A, G, P or L
  MISC_FEATURE (165)..(165): Xaa represents D, E, G, Q or N
  MISC_FEATURE (188)..(188): Xaa represents I, P, V or Y
SKYGPPXPPXPAPXAXGGPSVFLFPPKPKDTLMISRTPEVTCVVVDVSQEDPEVQFNWYVDGVEVHNAKTKPREEQFXSTYRVVSVLTVLHQDWLXGKEYKCKVSNKGLPSSIEKTISKAKGQPREPQVYTLPPSQEEMTKNQVSLXCXVKGFYPSDIAVEWESXGQPENNYKTTPPVLDSDGSFFLXSRLTVDKSRWQEGNVFSCSVMHEALHNHYTQKSLSLSLGK

SEQ ID NO: 3 - DNA, 1352 bp, Artificial Sequence
  Nucleotide sequence of first variant
tctagaaataattttgtttaactttaagaaggagatataccatgagcttcccgaccatcccgctgtctcgtctgttcgacaacgctatgctgcgtgctcaccgtctgcaccagctggcgttcgacacctaccaggaatttgaagaagcttacatcccgaaagaacagaaatactctttcctgcagaacccgcagacctctctgtgcttctctgaatctatcccgaccccgtctaaccgtgaagaaacccagcagaaatctaacctggaactgctgcgtatctctctgctgctgatccagtcttggctggaaccggttcagttcctgcgttctgttttcgctaactctctggtttacggtgcttctgactctaacgtttacgacctgctgaaagacctggaagaaggtatccagaccctgatgggtcgtctggaagacggttctccgcgtaccggtcagatcttcaaacagacctactctaaattcgacaccaactctcacaacgacgacgctctgctgaaaaactacggtctgctgtactgcttccgtaaagacatggacaaagttgaaaccttcctgcgtatcgttcagtgccgttctgttgaaggttcttgcggtttcggagcacctcagggtgctccacaaggcgcgccgcaaagcaaatacggcccgccatgtccaccgtgtccagcaccgaaggctgaaggcggtccgtctgtttttctgtttccgccgaaaccgaaagacaccctgatgattagtcgtaccccggaagttacctgcgttgttgttgacgtcagccaggaagatccggaagttcagttcaactggtacgttgacggcgttgaagttcataacgcgaaaaccaaaccgcgcgaagaacagttcaacagtacctatcgcgttgttagcgtactgaccgttctgcatcaggattggctgaacggcaaagagtacaaatgcaaagtcagcaacaaaggcctgccgagcagcattgaaaaaaccatcagcaaagcgaaaggccaaccgcgcgaaccgcaagtttataccctgccgccgtctcaggaagaaatgaccaaaaaccaggtcagcctgtggtgtctggttaaaggcttctacccgagcgatatcgcagttgagtgggaaagtaacggtcaaccggagaacaactataaaaccaccccgccggttctggatagcgacggtagctttttcctgtacagtcgtctgaccgttgataaaagccgttggcaggaaggcaacgtttttagctgtagcgtcatgcacgaagccctgcataaccattacacccagaaaagcctgagcctgagtctgggtaaataataaggatcc

SEQ ID NO: 4 - DNA, 740 bp, Artificial Sequence
  Nucleotide sequence of second variant
tctagaaataattttgtttaactttaagaaggagatataccatgtctaaatacggcccgccatgtccaccgtgtccagcaccggaggctaaaggtggtccgagcgtgttcctgtttccaccgaaaccgaaagataccctgatgatttctcgtactccggaggtaacttgcgtagtagttgatgtgagccaggaagatccggaggtgcagttcaactggtatgttgacggtgttgaggttcataacgccaagactaaaccacgtgaagaacagttccaaagcacctaccgtgtggtaagcgtgctgaccgttctgcaccaagattggctgcaaggtaaggagtacaaatgtaaagtaagcaacaaaggcctgccgagcagcattgagaagaccatctctaaggctaaaggtcaaccacgcgagccgcaggtgtacactctgccaccaagccaggaagagatgaccaagaatcaggtgtctctgagttgtgcagttaagggtttctacccgagcgatattgcggtagaatgggaatctcaaggtcagccggagaacaactataagaccactccaccagttctggattccgacggctctttcttcctggtatcccgtctgaccgttgacaaatcccgttggcaggaaggcaacgtgttctcttgttctgttatgcacgaggcgctgcacaaccactacacccagaagtctctgtccctgagcctgggtaaataataaggatcc

SEQ ID NO: 5 - protein, 432 aa, Artificial Sequence
  Amino acid sequence encoded by first variant
SFPTIPLSRLFDNAMLRAHRLHQLAFDTYQEFEEAYIPKEQKYSFLQNPQTSLCFSESIPTPSNREETQQKSNLELLRISLLLIQSWLEPVQFLRSVFANSLVYGASDSNVYDLLKDLEEGIQTLMGRLEDGSPRTGQIFKQTYSKFDTNSHNDDALLKNYGLLYCFRKDMDKVETFLRIVQCRSVEGSCGFGAPQGAPQGAPQSKYGPPCPPCPAPKAEGGPSVFLFPPKPKDTLMISRTPEVTCVVVDVSQEDPEVQFNWYVDGVEVHNAKTKPREEQFNSTYRVVSVLTVLHQDWLNGKEYKCKVSNKGLPSSIEKTISKAKGQPREPQVYTLPPSQEEMTKNQVSLWCLVKGFYPSDIAVEWESNGQPENNYKTTPPVLDSDGSFFLYSRLTVDKSRWQEGNVFSCSVMHEALHNHYTQKSLSLSLGK

SEQ ID NO: 6 - protein, 228 aa, Artificial Sequence
  Amino acid sequence encoded by second variant
SKYGPPCPPCPAPEAKGGPSVFLFPPKPKDTLMISRTPEVTCVVVDVSQEDPEVQFNWYVDGVEVHNAKTKPREEQFQSTYRVVSVLTVLHQDWLQGKEYKCKVSNKGLPSSIEKTISKAKGQPREPQVYTLPPSQEEMTKNQVSLSCAVKGFYPSDIAVEWESQGQPENNYKTTPPVLDSDGSFFLVSRLTVDKSRWQEGNVFSCSVMHEALHNHYTQKSLSLSLGK